European Patent Specification EP 3 442 559 B1, published May 1, 2024. Title: METHOD FOR THE TREATMENT OR PREVENTION OF OSTEOARTHRITIS. Applicant: Universiteit Maastricht and Academisch Ziekenhuis Maastricht. The sequence listing filed with the application follows.

SEQUENCE LISTING (64 sequences)

SEQ ID NO: 1 - protein, 47 aa, Homo sapiens
FINPETVPKPSSAPTQLNAISVLYFDDSSNVILKKYRNMVVRASGSH

SEQ ID NO: 2 - protein, 20 aa, Homo sapiens
FINPETVPKPSSAPTQLNAI

SEQ ID NO: 3 - protein, 20 aa, Homo sapiens
NPETVPKPSSAPTQLNAISV

SEQ ID NO: 4 - protein, 20 aa, Homo sapiens
ETVPKPSSAPTQLNAISVLY

SEQ ID NO: 5 - protein, 20 aa, Homo sapiens
VPKPSSAPTQLNAISVLYFD

SEQ ID NO: 6 - protein, 20 aa, Homo sapiens
PKPSSAPTQLNAISVLYFDD

SEQ ID NO: 7 - protein, 20 aa, Homo sapiens
KPSSAPTQLNAISVLYFDDS

SEQ ID NO: 8 - protein, 20 aa, Homo sapiens
SSAPTQLNAISVLYFDDSSN

SEQ ID NO: 9 - protein, 20 aa, Homo sapiens
APTQLNAISVLYFDDSSNVI

SEQ ID NO: 10 - protein, 20 aa, Homo sapiens
TQLNAISVLYFDDSSNVILK

SEQ ID NO: 11 - protein, 20 aa, Homo sapiens
LNAISVLYFDDSSNVILKKY

SEQ ID NO: 12 - protein, 20 aa, Homo sapiens
AISVLYFDDSSNVILKKYRN

SEQ ID NO: 13 - protein, 20 aa, Homo sapiens
SVLYFDDSSNVILKKYRNMV

SEQ ID NO: 14 - protein, 20 aa, Homo sapiens
LYFDDSSNVILKKYRNMVVR

SEQ ID NO: 15 - protein, 20 aa, Homo sapiens
FDDSSNVILKKYRNMVVRAS

SEQ ID NO: 16 - protein, 20 aa, Homo sapiens
DSSNVILKKYRNMVVRASGS

SEQ ID NO: 17 - protein, 20 aa, Homo sapiens
SSNVILKKYRNMVVRASGSH

SEQ ID NO: 18 - protein, 40 aa, Homo sapiens
PKPSSAPTQLNAISVLYFDDSSNVILKKYRNMVVRASGSH

SEQ ID NO: 19 - protein, 20 aa, Homo sapiens
STGSKQRSQNRSKTPKNQEA

SEQ ID NO: 20 - protein, 30 aa, Homo sapiens
KTPKNQEALRMANVAENSSSSSDQRQACKK

SEQ ID NO: 21 - protein, 20 aa, Homo sapiens
SSDQRQACKKHELYVSFRDL

SEQ ID NO: 22 - protein, 20 aa, Homo sapiens
DLGWQDWIIAPEGYAAYYCE

SEQ ID NO: 23 - protein, 20 aa, Homo sapiens
CEGECAFPLNSYMNATNHAI

SEQ ID NO: 24 - protein, 20 aa, Homo sapiens
AIVQTLVHFINPETVPKPCC

SEQ ID NO: 25 - protein, 20 aa, Homo sapiens
CCAPTQLNAISVLYFDDSSN

SEQ ID NO: 26 - protein, 20 aa, Homo sapiens
SSNVILKKYRNMVVRACGCH

SEQ ID NO: 27 - protein, 139 aa, Homo sapiens
STGSKQRSQNRSKTPKNQEALRMANVAENSSSDQRQACKKHELYVSFRDLGWQDWIIAPEGYAAYYCEGECAFPLNSYMNATNHAIVQTLVHFINPETVPKPCCAPTQLNAISVLYFDDSSNVILKKYRNMVVRACGCH

SEQ ID NO: 28 - protein, 139 aa, Homo sapiens
STGSKQRSQNRSKTPKNQEALRMANVAENSSSDQRQASKKHELYVSFRDLGWQDWIIAPEGYAAYYSEGESAFPLNSYMNATNHAIVQTLVHFINPETVPKPSSAPTQLNAISVLYFDDSSNVILKKYRNMVVRASGSH

SEQ ID NO: 29 - protein, 40 aa, Homo sapiens
  misc_feature (6)..(6): Xaa can be any naturally occurring amino acid
  misc_feature (8)..(9): Xaa can be any naturally occurring amino acid
  misc_feature (11)..(12): Xaa can be any naturally occurring amino acid
  misc_feature (14)..(14): Xaa can be any naturally occurring amino acid
  misc_feature (16)..(18): Xaa can be any naturally occurring amino acid
  misc_feature (20)..(31): Xaa can be any naturally occurring amino acid
  misc_feature (35)..(36): Xaa can be any naturally occurring amino acid
  misc_feature (40)..(40): Xaa can be any naturally occurring amino acid
PKPSSXPXXLXXIXVXXXDXXXXXXXXXXXXMVVXXSGSX

SEQ ID NO: 30 - protein, 12 aa, Homo sapiens
YSEGESAFPLNS

SEQ ID NO: 31 - protein, 12 aa, Homo sapiens
  misc_feature (5)..(5): Xaa can be any naturally occurring amino acid
  misc_feature (7)..(9): Xaa can be any naturally occurring amino acid
  misc_feature (11)..(12): Xaa can be any naturally occurring amino acid
YSEGXSXXXLXX

SEQ ID NO: 32 - protein, 28 aa, Homo sapiens
APEGYAAYYSEGESAFPLNSYMNATNHA

SEQ ID NO: 33 - protein, 28 aa, Homo sapiens
  misc_feature (1)..(3): Xaa can be any naturally occurring amino acid
  misc_feature (6)..(6): Xaa can be any naturally occurring amino acid
  misc_feature (8)..(8): Xaa can be any naturally occurring amino acid
  misc_feature (13)..(13): Xaa can be any naturally occurring amino acid
  misc_feature (15)..(17): Xaa can be any naturally occurring amino acid
  misc_feature (19)..(21): Xaa can be any naturally occurring amino acid
  misc_feature (26)..(26): Xaa can be any naturally occurring amino acid
XXXGYXAXYSEGXSXXXLXXXMNATXHA

SEQ ID NO: 34 - protein, 20 aa, Homo sapiens
APEGYAAYYSEGESAFPLNS

SEQ ID NO: 35 - protein, 20 aa, Homo sapiens
PEGYAAYYSEGESAFPLNSY

SEQ ID NO: 36 - protein, 20 aa, Homo sapiens
EGYAAYYSEGESAFPLNSYM

SEQ ID NO: 37 - protein, 20 aa, Homo sapiens
GYAAYYSEGESAFPLNSYMN

SEQ ID NO: 38 - protein, 20 aa, Homo sapiens
YAAYYSEGESAFPLNSYMNA

SEQ ID NO: 39 - protein, 20 aa, Homo sapiens
AAYYSEGESAFPLNSYMNAT

SEQ ID NO: 40 - protein, 20 aa, Homo sapiens
AYYSEGESAFPLNSYMNATN

SEQ ID NO: 41 - protein, 20 aa, Homo sapiens
YYSEGESAFPLNSYMNATNH

SEQ ID NO: 42 - protein, 20 aa, Homo sapiens
YSEGESAFPLNSYMNATNHA

SEQ ID NO: 43 - protein, 12 aa, Homo sapiens
YSEGESAFPLNS

SEQ ID NO: 44 - protein, 20 aa, Homo sapiens
APEGYAAYYSEGESAFPLNS

SEQ ID NO: 45 - protein, 19 aa, Homo sapiens
PEGYAAYYSEGESAFPLNS

SEQ ID NO: 46 - protein, 18 aa, Homo sapiens
EGYAAYYSEGESAFPLNS

SEQ ID NO: 47 - protein, 17 aa, Homo sapiens
GYAAYYSEGESAFPLNS

SEQ ID NO: 48 - protein, 16 aa, Homo sapiens
YAAYYSEGESAFPLNS

SEQ ID NO: 49 - protein, 20 aa, Homo sapiens
SFILKKVLYDRVNDSANIYS

SEQ ID NO: 50 - protein, 15 aa, Homo sapiens
AAYYSEGESAFPLNS

SEQ ID NO: 51 - protein, 14 aa, Homo sapiens
AYYSEGESAFPLNS

SEQ ID NO: 52 - protein, 13 aa, Homo sapiens
YYSEGESAFPLNS

SEQ ID NO: 53 - protein, 12 aa, Homo sapiens
YSEGESAFPLNS

SEQ ID NO: 54 - protein, 13 aa, Homo sapiens
YSEGESAFPLNSY

SEQ ID NO: 55 - protein, 14 aa, Homo sapiens
YSEGESAFPLNSYM

SEQ ID NO: 56 - protein, 15 aa, Homo sapiens
YSEGESAFPLNSYMN

SEQ ID NO: 57 - protein, 16 aa, Homo sapiens
YSEGESAFPLNSYMNA

SEQ ID NO: 58 - protein, 17 aa, Homo sapiens
YSEGESAFPLNSYMNAT

SEQ ID NO: 59 - protein, 18 aa, Homo sapiens
YSEGESAFPLNSYMNATN

SEQ ID NO: 60 - protein, 19 aa, Homo sapiens
YSEGESAFPLNSYMNATNH

SEQ ID NO: 61 - protein, 20 aa, Homo sapiens
YSEGESAFPLNSYMNATNHA

SEQ ID NO: 62 - protein, 28 aa, Homo sapiens
APEGYAAYYSEGESAFPLNSYMNATNHA

SEQ ID NO: 63 - protein, 27 aa, Homo sapiens
PEGYAAYYSEGESAFPLNSYMNATNHA

SEQ ID NO: 64 - protein, 26 aa, Homo sapiens
EGYAAYYSEGESAFPLNSYMNATNHA